European Patent Application EP 4 253 418 A1, published October 4, 2023. Title: IMMUNE CELLS EXPRESSING CHIMERIC ANTIGEN RECEPTORS AND BISPECIFIC ANTIBODIES AND USES THEREOF. Applicant: FUNDACIÓ PRIVADA INSTITUT D'INVESTIGACIÓ ONCOLÒGICA DE VALL HEBRON FUNDACIÓ INSTITUT MAR D'INVESTIGACIONS MÈDIQUES INSTITUCIÓ CATALANA DE RECERCA I ESTUDIS AVANÇATS. The sequence listing filed with the application follows.

SEQUENCE LISTING (101 sequences)

SEQ ID NO: 1 - protein, 5 aa, Artificial Sequence
  VH CDR1 ScFV anti-HER2
DTYIH

SEQ ID NO: 2 - protein, 17 aa, Artificial Sequence
  VH CDR2 ScFV anti-HER2
RIYPTNGYTRYADSVKG

SEQ ID NO: 3 - protein, 11 aa, Artificial Sequence
  VH CDR3 ScFV anti-HER2
WGGDGFYAMDV

SEQ ID NO: 4 - protein, 9 aa, Artificial Sequence
  VL CDR1 ScFV anti-HER2
RASQDVNTA

SEQ ID NO: 5 - protein, 8 aa, Artificial Sequence
  Target sequence of anti-p95HER2
PIWKFPDE

SEQ ID NO: 6 - protein, 9 aa, Artificial Sequence
  VL CDR3 ScFV anti-HER2
QQHYTTPPT

SEQ ID NO: 7 - protein, 5 aa, Artificial Sequence
  VH CDR1 ScFV anti-CD3
RYTMH

SEQ ID NO: 8 - protein, 17 aa, Artificial Sequence
  VH CDR2 ScFV anti-CD3
YINPSRGYTNYNQKFKD

SEQ ID NO: 9 - protein, 10 aa, Artificial Sequence
  VH CDR3 ScFV anti-CD3
YYDDHYCLDY

SEQ ID NO: 10 - protein, 10 aa, Artificial Sequence
  VL CDR1 ScFV anti-CD3
RASSSVSYMN

SEQ ID NO: 11 - protein, 642 aa, Homo sapiens
MPIWKFPDEEGACQPCPINCTHSCVDLDDKGCPAEQRASPLTSIISAVVGILLVVVLGVVFGILIKRRQQKIRKYTMRRLLQETELVEPLTPSGAMPNQAQMRILKETELRKVKVLGSGAFGTVYKGIWIPDGENVKIPVAIKVLRENTSPKANKEILDEAYVMAGVGSPYVSRLLGICLTSTVQLVTQLMPYGCLLDHVRENRGRLGSQDLLNWCMQIAKGMSYLEDVRLVHRDLAARNVLVKSPNHVKITDFGLARLLDIDETEYHADGGKVPIKWMALESILRRRFTHQSDVWSYGVTVWELTFGAKPYDGIPAREIPDLLEKGERLPQPPICTIDVYMIMVCWMIDSECRPRFRELVSEFSRMARDPQRFVVIQNEDLGPASPLDSTFYRSLLEDDDMGDLVDAEEYLVPQQGFFCPDPAPGAGGMVHHRHRSSSTRSGGGDLTLGLEPSEEEAPRSPLAPSEGAGSDVFDGDLGMGAAKGLQSLPTHDPSPLQRYSEDPTVPLPSETDGYVAPLTCSPQPEYVNQPDVRPQPPSPREGPLPAARPAGATLERPKTLSPGKNGVVKDFAFGGAVENPEYLTPQGGAAPQPHPPPAFSPAFDNLYYWDQDPPERGAPPSTFKGTPTAENPEYLGLDVPV

SEQ ID NO: 12 - protein, 9 aa, Artificial Sequence
  VL CDR3 ScFV anti-CD3
QQWSSNPLT

SEQ ID NO: 13 - protein, 30 aa, Artificial Sequence
  VH FR1 ScFV anti-HER2
EVQLVESGGGLVQPGGSLRLSCAASGFNIK

SEQ ID NO: 14 - protein, 14 aa, Artificial Sequence
  VH FR2 ScFV anti-HER2
WVRQAPGKGLEWVA

SEQ ID NO: 15 - protein, 32 aa, Artificial Sequence
  VH FR3 ScFV anti-HER2
RFTISADTSKNTAYLQMNSLRAEDTAVYYCSR

SEQ ID NO: 16 - protein, 11 aa, Artificial Sequence
  VH FR4 ScFV anti-HER2
WGQGTLVTVSS

SEQ ID NO: 17 - protein, 23 aa, Artificial Sequence
  VL FR1 ScFV anti-HER2
DIQMTQSPSSLSASVGDRVTITC

SEQ ID NO: 18 - protein, 17 aa, Artificial Sequence
  VL FR2 ScFV anti-HER2
VAWYQQKPGKAPKLLIY

SEQ ID NO: 19 - protein, 32 aa, Artificial Sequence
  VL FR3 ScFV anti-HER2
GVPSRFSGSRSGTDFTLTISSLQPEDFATYYC

SEQ ID NO: 20 - protein, 11 aa, Artificial Sequence
  VL FR4 ScFV anti-HER2
FGQGTKVEIKR

SEQ ID NO: 21 - protein, 30 aa, Artificial Sequence
  VH FR1 ScFV anti-CD3
DIKLQQSGAELARPGASVKMSCKTSGYTFT

SEQ ID NO: 22 - protein, 14 aa, Artificial Sequence
  VH FR2 ScFV anti-CD3
WVKQRPGQGLEWIG

SEQ ID NO: 23 - protein, 32 aa, Artificial Sequence
  VH FR3 ScFV anti-CD3
KATLTTDKSSSTAYMQLSSLTSEDSAVYYCAR

SEQ ID NO: 24 - protein, 13 aa, Artificial Sequence
  VH FR4 ScFV anti-CD3
WGQGTTLTVSSVE

SEQ ID NO: 25 - protein, 23 aa, Artificial Sequence
  VL FR1 ScFV anti-CD3
DIQLTQSPAIMSASPGEKVTMTC

SEQ ID NO: 26 - protein, 15 aa, Artificial Sequence
  VL FR2 ScFV anti-CD3
WYQQKSGTSPKRWIY

SEQ ID NO: 27 - protein, 32 aa, Artificial Sequence
  VL FR3 ScFV anti-CD3
GVPYRFSGSGSGTSYSLTISSMEAEDAATYYC

SEQ ID NO: 28 - protein, 10 aa, Artificial Sequence
  VL FR4 ScFV anti-CD3
FGAGTKLELK

SEQ ID NO: 29 - protein, 120 aa, Artificial Sequence
  VH ScFv anti-HER2
EVQLVESGGGLVQPGGSLRLSCAASGFNIKDTYIHWVRQAPGKGLEWVARIYPTNGYTRYADSVKGRFTISADTSKNTAYLQMNSLRAEDTAVYYCSRWGGDGFYAMDVWGQGTLVTVSS

SEQ ID NO: 30 - protein, 108 aa, Artificial Sequence
  VL ScFv anti-HER2
DIQMTQSPSSLSASVGDRVTITCRASQDVNTAVAWYQQKPGKAPKLLIYSASFLYSGVPSRFSGSRSGTDFTLTISSLQPEDFATYYCQQHYTTPPTFGQGTKVEIKR

SEQ ID NO: 31 - protein, 121 aa, Artificial Sequence
  VH ScFV anti-CD3
DIKLQQSGAELARPGASVKMSCKTSGYTFTRYTMHWVKQRPGQGLEWIGYINPSRGYTNYNQKFKDKATLTTDKSSSTAYMQLSSLTSEDSAVYYCARYYDDHYCLDYWGQGTTLTVSSVE

SEQ ID NO: 32 - protein, 106 aa, Artificial Sequence
  VL ScFV anti-CD3
DIQLTQSPAIMSASPGEKVTMTCRASSSVSYMNWYQQKSGTSPKRWIYDTSKVASGVPYRFSGSGSGTSYSLTISSMEAEDAATYYCQQWSSNPLTFGAGTKLELK

SEQ ID NO: 33 - protein, 15 aa, Artificial Sequence
  Linker
GGGGSGGGGSGGGGS

SEQ ID NO: 34 - protein, 5 aa, Artificial Sequence
  Linker
GGGGS

SEQ ID NO: 35 - protein, 16 aa, Artificial Sequence
  Linker
GGSGGSGGSGGSGGVD

SEQ ID NO: 36 - protein, 243 aa, Artificial Sequence
  ScFv anti-HER2
DIQMTQSPSSLSASVGDRVTITCRASQDVNTAVAWYQQKPGKAPKLLIYSASFLYSGVPSRFSGSRSGTDFTLTISSLQPEDFATYYCQQHYTTPPTFGQGTKVEIKRGGGGSGGGGSGGGGSEVQLVESGGGLVQPGGSLRLSCAASGFNIKDTYIHWVRQAPGKGLEWVARIYPTNGYTRYADSVKGRFTISADTSKNTAYLQMNSLRAEDTAVYYCSRWGGDGFYAMDVWGQGTLVTVSS

SEQ ID NO: 37 - protein, 243 aa, Artificial Sequence
  ScFv anti-CD3
DIKLQQSGAELARPGASVKMSCKTSGYTFTRYTMHWVKQRPGQGLEWIGYINPSRGYTNYNQKFKDKATLTTDKSSSTAYMQLSSLTSEDSAVYYCARYYDDHYCLDYWGQGTTLTVSSVEGGSGGSGGSGGSGGVDDIQLTQSPAIMSASPGEKVTMTCRASSSVSYMNWYQQKSGTSPKRWIYDTSKVASGVPYRFSGSGSGTSYSLTISSMEAEDAATYYCQQWSSNPLTFGAGTKLELK

SEQ ID NO: 38 - protein, 491 aa, Artificial Sequence
  HER2-CD3 BiTE
DIQMTQSPSSLSASVGDRVTITCRASQDVNTAVAWYQQKPGKAPKLLIYSASFLYSGVPSRFSGSRSGTDFTLTISSLQPEDFATYYCQQHYTTPPTFGQGTKVEIKRGGGGSGGGGSGGGGSEVQLVESGGGLVQPGGSLRLSCAASGFNIKDTYIHWVRQAPGKGLEWVARIYPTNGYTRYADSVKGRFTISADTSKNTAYLQMNSLRAEDTAVYYCSRWGGDGFYAMDVWGQGTLVTVSSGGGGSDIKLQQSGAELARPGASVKMSCKTSGYTFTRYTMHWVKQRPGQGLEWIGYINPSRGYTNYNQKFKDKATLTTDKSSSTAYMQLSSLTSEDSAVYYCARYYDDHYCLDYWGQGTTLTVSSVEGGSGGSGGSGGSGGVDDIQLTQSPAIMSASPGEKVTMTCRASSSVSYMNWYQQKSGTSPKRWIYDTSKVASGVPYRFSGSGSGTSYSLTISSMEAEDAATYYCQQWSSNPLTFGAGTKLELK

SEQ ID NO: 39 - protein, 5 aa, Artificial Sequence
  VH CDR1 214 (214D8)
TYGMA

SEQ ID NO: 40 - protein, 17 aa, Artificial Sequence
  VH CDR2 214 (214D8)
TINSNGGKTYHPDSVKG

SEQ ID NO: 41 - protein, 5 aa, Artificial Sequence
  VH CDR3 214 (214D8)
EGFDY

SEQ ID NO: 42 - protein, 11 aa, Artificial Sequence
  VL CDR1 214 (214D8)
KASQNVGTAVA

SEQ ID NO: 43 - protein, 7 aa, Artificial Sequence
  VL CDR2 214 (214D8)
SASNRYT

SEQ ID NO: 44 - protein, 9 aa, Artificial Sequence
  VL CDR3 214 (214D8)
QQYSTYPLT

SEQ ID NO: 45 - protein, 30 aa, Artificial Sequence
  VH FR1 H1-214
EVQLVESGGGLVQPGGSLRLSCAASGFTFS

SEQ ID NO: 46 - protein, 14 aa, Artificial Sequence
  VH FR2 H1-214
WVRQTPDRRLELVA

SEQ ID NO: 47 - protein, 32 aa, Artificial Sequence
  VH FR3 H1-214
RFTISRDNSKNTLYLQMNSLRAEDTAVYYCTR

SEQ ID NO: 48 - protein, 11 aa, Artificial Sequence
  VH FR4 H1-214
WGQGTLVTVSS

SEQ ID NO: 49 - protein, 23 aa, Artificial Sequence
  VL FR1 H1-214
DIQMTQSPSSLSASVGDRVTITC

SEQ ID NO: 50 - protein, 15 aa, Artificial Sequence
  VL FR2 H1-214
WFQQKPGKAPKILIY

SEQ ID NO: 51 - protein, 32 aa, Artificial Sequence
  VL FR3 H1-214
GVPSRFSGSGSGTDFTLTISSLQPEDFATYYC

SEQ ID NO: 52 - protein, 10 aa, Artificial Sequence
  VL FR4 H1-214
FGQGTKLEIK

SEQ ID NO: 53 - protein, 16 aa, Artificial Sequence
  Linker region
TGSTSGSGKPGSGEGS

SEQ ID NO: 54 - protein, 107 aa, Artificial Sequence
  VL CAR
DIQMTQSPSSLSASVGDRVTITCKASQNVGTAVAWFQQKPGKAPKILIYSASNRYTGVPSRFSGSGSGTDFTLTISSLQPEDFATYYCQQYSTYPLTFGQGTKLEIK

SEQ ID NO: 55 - protein, 114 aa, Artificial Sequence
  VH CAR
EVQLVESGGGLVQPGGSLRLSCAASGFTFSTYGMAWVRQTPDRRLELVATINSNGGKTYHPDSVKGRFTISRDNSKNTLYLQMNSLRAEDTAVYYCTREGFDYWGQGTLVTVSS

SEQ ID NO: 56 - protein, 237 aa, Artificial Sequence
  CAR SvFv
DIQMTQSPSSLSASVGDRVTITCKASQNVGTAVAWFQQKPGKAPKILIYSASNRYTGVPSRFSGSGSGTDFTLTISSLQPEDFATYYCQQYSTYPLTFGQGTKLEIKTGSTSGSGKPGSGEGSEVQLVESGGGLVQPGGSLRLSCAASGFTFSTYGMAWVRQTPDRRLELVATINSNGGKTYHPDSVKGRFTISRDNSKNTLYLQMNSLRAEDTAVYYCTREGFDYWGQGTLVTVSS

SEQ ID NO: 57 - protein, 27 aa, Artificial Sequence
  FWVLVVVGGVLACYSLLVTVAFIIFWV
FWVLVVVGGVLACYSLLVTVAFIIFWV

SEQ ID NO: 58 - protein, 41 aa, Artificial Sequence
  CD28 costimulatory domain
RSKRSRLLHSDYMNMTPRRPGPTRKHYQPYAPPRDFAAYRS

SEQ ID NO: 59 - protein, 112 aa, Artificial Sequence
  CD3-zeta intracellular signalling domain
RVKFSRSADAPAYQQGQNQLYNELNLGRREEYDVLDKRRGRDPEMGGKPRRKNPQEGLYNELQKDKMAEAYSEIGMKGERRRGKGHDGLYQGLSTATKDTYDALHMQALPPR

SEQ ID NO: 60 - protein, 45 aa, Artificial Sequence
  CD8 hinge region
TTTPAPRPPTPAPTIASQPLSLRPEACRPAAGGAVHTRGLDFACD

SEQ ID NO: 61 - protein, 462 aa, Artificial Sequence
  Complete CAR
DIQMTQSPSSLSASVGDRVTITCKASQNVGTAVAWFQQKPGKAPKILIYSASNRYTGVPSRFSGSGSGTDFTLTISSLQPEDFATYYCQQYSTYPLTFGQGTKLEIKTGSTSGSGKPGSGEGSEVQLVESGGGLVQPGGSLRLSCAASGFTFSTYGMAWVRQTPDRRLELVATINSNGGKTYHPDSVKGRFTISRDNSKNTLYLQMNSLRAEDTAVYYCTREGFDYWGQGTLVTVSSTTTPAPRPPTPAPTIASQPLSLRPEACRPAAGGAVHTRGLDFACDFWVLVVVGGVLACYSLLVTVAFIIFWVRSKRSRLLHSDYMNMTPRRPGPTRKHYQPYAPPRDFAAYRSRVKFSRSADAPAYQQGQNQLYNELNLGRREEYDVLDKRRGRDPEMGGKPRRKNPQEGLYNELQKDKMAEAYSEIGMKGERRRGKGHDGLYQGLSTATKDTYDALHMQALPPR

SEQ ID NO: 62 - protein, 21 aa, Artificial Sequence
  Signal sequence CD8a
MALPVTALLLPLALLLHAARP

SEQ ID NO: 63 - protein, 22 aa, Artificial Sequence
  Signal sequence IgK
MDFQVQIFSFLLISASVIMSRG

SEQ ID NO: 64 - protein, 18 aa, Artificial Sequence
  Self-cleaving peptide
EGRGSLLTCGDVEENPGP

SEQ ID NO: 65 - protein, 1014 aa, Artificial Sequence
  CAR-BITE (sin 6xHis tag)
MALPVTALLLPLALLLHAARPDIQMTQSPSSLSASVGDRVTITCKASQNVGTAVAWFQQKPGKAPKILIYSASNRYTGVPSRFSGSGSGTDFTLTISSLQPEDFATYYCQQYSTYPLTFGQGTKLEIKTGSTSGSGKPGSGEGSEVQLVESGGGLVQPGGSLRLSCAASGFTFSTYGMAWVRQTPDRRLELVATINSNGGKTYHPDSVKGRFTISRDNSKNTLYLQMNSLRAEDTAVYYCTREGFDYWGQGTLVTVSSTTTPAPRPPTPAPTIASQPLSLRPEACRPAAGGAVHTRGLDFACDFWVLVVVGGVLACYSLLVTVAFIIFWVRSKRSRLLHSDYMNMTPRRPGPTRKHYQPYAPPRDFAAYRSRVKFSRSADAPAYQQGQNQLYNELNLGRREEYDVLDKRRGRDPEMGGKPRRKNPQEGLYNELQKDKMAEAYSEIGMKGERRRGKGHDGLYQGLSTATKDTYDALHMQALPPREGRGSLLTCGDVEENPGPMDFQVQIFSFLLISASVIMSRGDIQMTQSPSSLSASVGDRVTITCRASQDVNTAVAWYQQKPGKAPKLLIYSASFLYSGVPSRFSGSRSGTDFTLTISSLQPEDFATYYCQQHYTTPPTFGQGTKVEIKRGGGGSGGGGSGGGGSEVQLVESGGGLVQPGGSLRLSCAASGFNIKDTYIHWVRQAPGKGLEWVARIYPTNGYTRYADSVKGRFTISADTSKNTAYLQMNSLRAEDTAVYYCSRWGGDGFYAMDVWGQGTLVTVSSGGGGSDIKLQQSGAELARPGASVKMSCKTSGYTFTRYTMHWVKQRPGQGLEWIGYINPSRGYTNYNQKFKDKATLTTDKSSSTAYMQLSSLTSEDSAVYYCARYYDDHYCLDYWGQGTTLTVSSVEGGSGGSGGSGGSGGVDDIQLTQSPAIMSASPGEKVTMTCRASSSVSYMNWYQQKSGTSPKRWIYDTSKVASGVPYRFSGSGSGTSYSLTISSMEAEDAATYYCQQWSSNPLTFGAGTKLELK

SEQ ID NO: 66 - protein, 1020 aa, Artificial Sequence
  CAR-BITE (con 6xHis tag)
MALPVTALLLPLALLLHAARPDIQMTQSPSSLSASVGDRVTITCKASQNVGTAVAWFQQKPGKAPKILIYSASNRYTGVPSRFSGSGSGTDFTLTISSLQPEDFATYYCQQYSTYPLTFGQGTKLEIKTGSTSGSGKPGSGEGSEVQLVESGGGLVQPGGSLRLSCAASGFTFSTYGMAWVRQTPDRRLELVATINSNGGKTYHPDSVKGRFTISRDNSKNTLYLQMNSLRAEDTAVYYCTREGFDYWGQGTLVTVSSTTTPAPRPPTPAPTIASQPLSLRPEACRPAAGGAVHTRGLDFACDFWVLVVVGGVLACYSLLVTVAFIIFWVRSKRSRLLHSDYMNMTPRRPGPTRKHYQPYAPPRDFAAYRSRVKFSRSADAPAYQQGQNQLYNELNLGRREEYDVLDKRRGRDPEMGGKPRRKNPQEGLYNELQKDKMAEAYSEIGMKGERRRGKGHDGLYQGLSTATKDTYDALHMQALPPREGRGSLLTCGDVEENPGPMDFQVQIFSFLLISASVIMSRGDIQMTQSPSSLSASVGDRVTITCRASQDVNTAVAWYQQKPGKAPKLLIYSASFLYSGVPSRFSGSRSGTDFTLTISSLQPEDFATYYCQQHYTTPPTFGQGTKVEIKRGGGGSGGGGSGGGGSEVQLVESGGGLVQPGGSLRLSCAASGFNIKDTYIHWVRQAPGKGLEWVARIYPTNGYTRYADSVKGRFTISADTSKNTAYLQMNSLRAEDTAVYYCSRWGGDGFYAMDVWGQGTLVTVSSGGGGSDIKLQQSGAELARPGASVKMSCKTSGYTFTRYTMHWVKQRPGQGLEWIGYINPSRGYTNYNQKFKDKATLTTDKSSSTAYMQLSSLTSEDSAVYYCARYYDDHYCLDYWGQGTTLTVSSVEGGSGGSGGSGGSGGVDDIQLTQSPAIMSASPGEKVTMTCRASSSVSYMNWYQQKSGTSPKRWIYDTSKVASGVPYRFSGSGSGTSYSLTISSMEAEDAATYYCQQWSSNPLTFGAGTKLELKHHHHHH

SEQ ID NO: 67 - protein, 5 aa, Artificial Sequence
  linker region
GSGGS

SEQ ID NO: 68 - protein, 4 aa, Artificial Sequence
  linker region
GGGS

SEQ ID NO: 69 - protein, 4 aa, Artificial Sequence
  Flexible linker
GGSG

SEQ ID NO: 70 - protein, 5 aa, Artificial Sequence
  Flexible linker
GGSGG

SEQ ID NO: 71 - protein, 5 aa, Artificial Sequence
  Flexible linker
GSGSG

SEQ ID NO: 72 - protein, 5 aa, Artificial Sequence
  Flexible linker
GSGGG

SEQ ID NO: 73 - protein, 5 aa, Artificial Sequence
  Flexible linker
GGGSG

SEQ ID NO: 74 - protein, 5 aa, Artificial Sequence
  Flexible linker
GSSSG

SEQ ID NO: 75 - protein, 4 aa, Artificial Sequence
  Ig hinge domain
CPPC

SEQ ID NO: 76 - protein, 5 aa, Artificial Sequence
  Ig hinge domain
DKTHT

SEQ ID NO: 77 - protein, 15 aa, Artificial Sequence
  Ig hinge domain
CPEPKSCDTPPPCPR

SEQ ID NO: 78 - protein, 12 aa, Artificial Sequence
  Ig hinge domain
ELKTPLGDTTHT

SEQ ID NO: 79 - protein, 10 aa, Artificial Sequence
  Ig hinge domain
KSCDKTHTCP

SEQ ID NO: 80 - protein, 7 aa, Artificial Sequence
  Ig hinge domain
KCCVDCP

SEQ ID NO: 81 - protein, 7 aa, Artificial Sequence
  Ig hinge domain
KYGPPCP

SEQ ID NO: 82 - protein, 15 aa, Artificial Sequence
  Ig hinge domain
EPKSCDKTHTCPPCP

SEQ ID NO: 83 - protein, 12 aa, Artificial Sequence
  Ig hinge domain
ERKCCVECPPCP

SEQ ID NO: 84 - protein, 17 aa, Artificial Sequence
  Ig hinge domain
ELKTPLGDTTHTCPRCP

SEQ ID NO: 85 - protein, 12 aa, Artificial Sequence
  Ig hinge domain
SPNMVPHAHHAQ

SEQ ID NO: 86 - protein, 15 aa, Artificial Sequence
  Ig hinge domain
EPKSCDKTYTCPPCP

SEQ ID NO: 87 - protein, 22 aa, Artificial Sequence
  self-cleaving peptide
VKQTLNFDLLKLAGDVESNPGP

SEQ ID NO: 88 - protein, 20 aa, Artificial Sequence
  self-cleaving peptide
QCTNYALLKLAGDVESNPGP

SEQ ID NO: 89 - protein, 19 aa, Artificial Sequence
  self-cleaving peptide
ATNFSLLKQAGDVEENPGP

SEQ ID NO: 90 - protein, 63 aa, Artificial Sequence
  CHYSEL
GSGSRVTELLYRMKRAETYCPRPLLAIHPTEARHKQKIVAPVKQLLNFDLLKLAGDVESNPGP

SEQ ID NO: 91 - protein, 19 aa, Artificial Sequence
  CHYSEL
LLCFLLLLLSGDVELNPGP

SEQ ID NO: 92 - protein, 20 aa, Artificial Sequence
  CHYSEL
HHFMFLLLLLAGDIELNPGP

SEQ ID NO: 93 - protein, 20 aa, Artificial Sequence
  CHYSEL
WFLVLLSFILSGDIEVNPGP

SEQ ID NO: 94 - protein, 20 aa, Artificial Sequence
  CHYSEL
KNCAMYMLLLSGDVETNPGP

SEQ ID NO: 95 - protein, 20 aa, Artificial Sequence
  CHYSEL
MVISQLMLKLAGDVEENPGP

SEQ ID NO: 96 - protein, 22 aa, Artificial Sequence
  CHYSEL
GSGATNFSLLKQAGDVEENPGP

SEQ ID NO: 97 - protein, 21 aa, Artificial Sequence
  CHYSEL
GSGEGRGSLLTCGDVEENPGP

SEQ ID NO: 98 - protein, 23 aa, Artificial Sequence
  CHYSEL
GSGQCTNYALLKLAGDVESNPGP

SEQ ID NO: 99 - protein, 8 aa, Artificial Sequence
  CHYSEL
  misc_feature (2)..(2): Xaa can be any naturally occurring amino acid
  misc_feature (4)..(4): Xaa can be any naturally occurring amino acid
DXEXNPGP

SEQ ID NO: 100 - protein, 7 aa, Artificial Sequence
  VL CDR2
SASFLYS

SEQ ID NO: 101 - protein, 7 aa, Artificial Sequence
  Second Antigen bidning region VL CDR2
DTSKVAS